European Patent Application EP 4 571 310 A1, published June 18, 2025. Title: ｐ５３アイソフォーム変異体のがん診断用途. Applicant: YAMAHA HATSUDOKI KABUSHIKI KAISHA. The sequence listing filed with the application follows.

SEQUENCE LISTING (70 sequences)

SEQ ID NO: 1 - protein, 393 aa, Homo sapiens [sequence omitted]

SEQ ID NO: 2 - protein, 341 aa, Homo sapiens
MEEPQSDPSVEPPLSQETFSDLWKLLPENNVLSPLPSQAMDDLMLSPDDIEQWFTEDPGPDEAPRMPEAAPPVAPAPAAPTPAAPAPAPSWPLSSSVPSQKTYQGSYGFRLGFLHSGTAKSVTCTYSPALNKMFCQLAKTCPVQLWVDSTPPPGTRVRAMAIYKQSQHMTEVVRRCPHHERCSDSDGLAPPQHLIRVEGNLRVEYLDDRNTFRHSVVVPYEPPEVGSDCTTIHYNYMCNSSCMGGMNRRPILTIITLEDSSGNLLGRNSFEVRVCACPGRDRRTEEENLRKKGEPHHELPPGSTKRALPNNTSSSPQPKKKPLDGEYFTLQDQTSFQKENC

SEQ ID NO: 3 - protein, 346 aa, Homo sapiens
MEEPQSDPSVEPPLSQETFSDLWKLLPENNVLSPLPSQAMDDLMLSPDDIEQWFTEDPGPDEAPRMPEAAPPVAPAPAAPTPAAPAPAPSWPLSSSVPSQKTYQGSYGFRLGFLHSGTAKSVTCTYSPALNKMFCQLAKTCPVQLWVDSTPPPGTRVRAMAIYKQSQHMTEVVRRCPHHERCSDSDGLAPPQHLIRVEGNLRVEYLDDRNTFRHSVVVPYEPPEVGSDCTTIHYNYMCNSSCMGGMNRRPILTIITLEDSSGNLLGRNSFEVRVCACPGRDRRTEEENLRKKGEPHHELPPGSTKRALPNNTSSSPQPKKKPLDGEYFTLQMLLDLRWCYFLINSS

SEQ ID NO: 4 - protein, 354 aa, Homo sapiens
MDDLMLSPDDIEQWFTEDPGPDEAPRMPEAAPPVAPAPAAPTPAAPAPAPSWPLSSSVPSQKTYQGSYGFRLGFLHSGTAKSVTCTYSPALNKMFCQLAKTCPVQLWVDSTPPPGTRVRAMAIYKQSQHMTEVVRRCPHHERCSDSDGLAPPQHLIRVEGNLRVEYLDDRNTFRHSVVVPYEPPEVGSDCTTIHYNYMCNSSCMGGMNRRPILTIITLEDSSGNLLGRNSFEVRVCACPGRDRRTEEENLRKKGEPHHELPPGSTKRALPNNTSSSPQPKKKPLDGEYFTLQIRGRERFEMFRELNEALELKDAQAGKEPGGSRAHSSHLKSKKGQSTSRHKKLMFKTEGPDSD

SEQ ID NO: 5 - protein, 302 aa, Homo sapiens
MDDLMLSPDDIEQWFTEDPGPDEAPRMPEAAPPVAPAPAAPTPAAPAPAPSWPLSSSVPSQKTYQGSYGFRLGFLHSGTAKSVTCTYSPALNKMFCQLAKTCPVQLWVDSTPPPGTRVRAMAIYKQSQHMTEVVRRCPHHERCSDSDGLAPPQHLIRVEGNLRVEYLDDRNTFRHSVVVPYEPPEVGSDCTTIHYNYMCNSSCMGGMNRRPILTIITLEDSSGNLLGRNSFEVRVCACPGRDRRTEEENLRKKGEPHHELPPGSTKRALPNNTSSSPQPKKKPLDGEYFTLQDQTSFQKENC

SEQ ID NO: 6 - protein, 307 aa, Homo sapiens
MDDLMLSPDDIEQWFTEDPGPDEAPRMPEAAPPVAPAPAAPTPAAPAPAPSWPLSSSVPSQKTYQGSYGFRLGFLHSGTAKSVTCTYSPALNKMFCQLAKTCPVQLWVDSTPPPGTRVRAMAIYKQSQHMTEVVRRCPHHERCSDSDGLAPPQHLIRVEGNLRVEYLDDRNTFRHSVVVPYEPPEVGSDCTTIHYNYMCNSSCMGGMNRRPILTIITLEDSSGNLLGRNSFEVRVCACPGRDRRTEEENLRKKGEPHHELPPGSTKRALPNNTSSSPQPKKKPLDGEYFTLQMLLDLRWCYFLINSS

SEQ ID NO: 7 - protein, 261 aa, Homo sapiens
MFCQLAKTCPVQLWVDSTPPPGTRVRAMAIYKQSQHMTEVVRRCPHHERCSDSDGLAPPQHLIRVEGNLRVEYLDDRNTFRHSVVVPYEPPEVGSDCTTIHYNYMCNSSCMGGMNRRPILTIITLEDSSGNLLGRNSFEVRVCACPGRDRRTEEENLRKKGEPHHELPPGSTKRALPNNTSSSPQPKKKPLDGEYFTLQIRGRERFEMFRELNEALELKDAQAGKEPGGSRAHSSHLKSKKGQSTSRHKKLMFKTEGPDSD

SEQ ID NO: 8 - protein, 209 aa, Homo sapiens
MFCQLAKTCPVQLWVDSTPPPGTRVRAMAIYKQSQHMTEVVRRCPHHERCSDSDGLAPPQHLIRVEGNLRVEYLDDRNTFRHSVVVPYEPPEVGSDCTTIHYNYMCNSSCMGGMNRRPILTIITLEDSSGNLLGRNSFEVRVCACPGRDRRTEEENLRKKGEPHHELPPGSTKRALPNNTSSSPQPKKKPLDGEYFTLQDQTSFQKENC

SEQ ID NO: 9 - protein, 214 aa, Homo sapiens
MFCQLAKTCPVQLWVDSTPPPGTRVRAMAIYKQSQHMTEVVRRCPHHERCSDSDGLAPPQHLIRVEGNLRVEYLDDRNTFRHSVVVPYEPPEVGSDCTTIHYNYMCNSSCMGGMNRRPILTIITLEDSSGNLLGRNSFEVRVCACPGRDRRTEEENLRKKGEPHHELPPGSTKRALPNNTSSSPQPKKKPLDGEYFTLQMLLDLRWCYFLINSS

SEQ ID NO: 10 - protein, 234 aa, Homo sapiens
MAIYKQSQHMTEVVRRCPHHERCSDSDGLAPPQHLIRVEGNLRVEYLDDRNTFRHSVVVPYEPPEVGSDCTTIHYNYMCNSSCMGGMNRRPILTIITLEDSSGNLLGRNSFEVRVCACPGRDRRTEEENLRKKGEPHHELPPGSTKRALPNNTSSSPQPKKKPLDGEYFTLQIRGRERFEMFRELNEALELKDAQAGKEPGGSRAHSSHLKSKKGQSTSRHKKLMFKTEGPDSD

SEQ ID NO: 11 - protein, 182 aa, Homo sapiens
MAIYKQSQHMTEVVRRCPHHERCSDSDGLAPPQHLIRVEGNLRVEYLDDRNTFRHSVVVPYEPPEVGSDCTTIHYNYMCNSSCMGGMNRRPILTIITLEDSSGNLLGRNSFEVRVCACPGRDRRTEEENLRKKGEPHHELPPGSTKRALPNNTSSSPQPKKKPLDGEYFTLQDQTSFQKENC

SEQ ID NO: 12 - protein, 187 aa, Homo sapiens
MAIYKQSQHMTEVVRRCPHHERCSDSDGLAPPQHLIRVEGNLRVEYLDDRNTFRHSVVVPYEPPEVGSDCTTIHYNYMCNSSCMGGMNRRPILTIITLEDSSGNLLGRNSFEVRVCACPGRDRRTEEENLRKKGEPHHELPPGSTKRALPNNTSSSPQPKKKPLDGEYFTLQMLLDLRWCYFLINSS

SEQ ID NO: 13 - protein, 341 aa, Homo sapiens
MEEPQSDPSVEPPLSQETFSDLWKLLPENNVLSPLPSQAMDDLMLSPDDIEQWFTEDPGPDEAPRMPEAAPPVAPAPAAPTPAAPAPAPSWPLSSSVPSQKTYQGSYGFRLGFLHSGTAKSVTCTYSPALNKMFCQLAKTCPVQLWVDSTPPPGTRVRAMAIYKQSQHMTEVVRRCPHHERCSDSDGLAPPQHLIRVEGNLRVEYLDDRNTFRHSVVVPYEPPEVGSDCTTIHYNYMCNSSCMGGMNRRPILTIITLEDSSGNLLGRNSFEVRVCACPGRDRRTEEENLRKKGEPHHELPPGSTKRALPNNTSSSPQPKKKPLDGEYFTLQIRGRERFEMF

SEQ ID NO: 14 - protein, 330 aa, Homo sapiens
MEEPQSDPSVEPPLSQETFSDLWKLLPENNVLSPLPSQAMDDLMLSPDDIEQWFTEDPGPDEAPRMPEAAPPVAPAPAAPTPAAPAPAPSWPLSSSVPSQKTYQGSYGFRLGFLHSGTAKSVTCTYSPALNKMFCQLAKTCPVQLWVDSTPPPGTRVRAMAIYKQSQHMTEVVRRCPHHERCSDSDGLAPPQHLIRVEGNLRVEYLDDRNTFRHSVVVPYEPPEVGSDCTTIHYNYMCNSSCMGGMNRRPILTIITLEDSSGNLLGRNSFEVRVCACPGRDRRTEEENLRKKGEPHHELPPGSTKRALPNNTSSSPQPKKKPLDGEYFTL

SEQ ID NO: 15 - protein, 316 aa, Homo sapiens
MEEPQSDPSVEPPLSQETFSDLWKLLPENNVLSPLPSQAMDDLMLSPDDIEQWFTEDPGPDEAPRMPEAAPPVAPAPAAPTPAAPAPAPSWPLSSSVPSQKTYQGSYGFRLGFLHSGTAKSVTCTYSPALNKMFCQLAKTCPVQLWVDSTPPPGTRVRAMAIYKQSQHMTEVVRRCPHHERCSDSDGLAPPQHLIRVEGNLRVEYLDDRNTFRHSVVVPYEPPEVGSDCTTIHYNYMCNSSCMGGMNRRPILTIITLEDSSGNLLGRNSFEVRVCACPGRDRRTEEENLRKKGEPHHELPPGSTKRALPNNTSSSP

SEQ ID NO: 16 - protein, 305 aa, Homo sapiens
MEEPQSDPSVEPPLSQETFSDLWKLLPENNVLSPLPSQAMDDLMLSPDDIEQWFTEDPGPDEAPRMPEAAPPVAPAPAAPTPAAPAPAPSWPLSSSVPSQKTYQGSYGFRLGFLHSGTAKSVTCTYSPALNKMFCQLAKTCPVQLWVDSTPPPGTRVRAMAIYKQSQHMTEVVRRCPHHERCSDSDGLAPPQHLIRVEGNLRVEYLDDRNTFRHSVVVPYEPPEVGSDCTTIHYNYMCNSSCMGGMNRRPILTIITLEDSSGNLLGRNSFEVRVCACPGRDRRTEEENLRKKGEPHHELPPGSTK

SEQ ID NO: 17 - protein, 191 aa, Homo sapiens
MEEPQSDPSVEPPLSQETFSDLWKLLPENNVLSPLPSQAMDDLMLSPDDIEQWFTEDPGPDEAPRMPEAAPPVAPAPAAPTPAAPAPAPSWPLSSSVPSQKTYQGSYGFRLGFLHSGTAKSVTCTYSPALNKMFCQLAKTCPVQLWVDSTPPPGTRVRAMAIYKQSQHMTEVVRRCPHHERCSDSDGLAPP

SEQ ID NO: 18 - protein, 145 aa, Homo sapiens
MEEPQSDPSVEPPLSQETFSDLWKLLPENNVLSPLPSQAMDDLMLSPDDIEQWFTEDPGPDEAPRMPEAAPPVAPAPAAPTPAAPAPAPSWPLSSSVPSQKTYQGSYGFRLGFLHSGTAKSVTCTYSPALNKMFCQLAKTCPVQL

SEQ ID NO: 19 - protein, 302 aa, Homo sapiens
MDDLMLSPDDIEQWFTEDPGPDEAPRMPEAAPPVAPAPAAPTPAAPAPAPSWPLSSSVPSQKTYQGSYGFRLGFLHSGTAKSVTCTYSPALNKMFCQLAKTCPVQLWVDSTPPPGTRVRAMAIYKQSQHMTEVVRRCPHHERCSDSDGLAPPQHLIRVEGNLRVEYLDDRNTFRHSVVVPYEPPEVGSDCTTIHYNYMCNSSCMGGMNRRPILTIITLEDSSGNLLGRNSFEVRVCACPGRDRRTEEENLRKKGEPHHELPPGSTKRALPNNTSSSPQPKKKPLDGEYFTLQIRGRERFEMF

SEQ ID NO: 20 - protein, 291 aa, Homo sapiens
MDDLMLSPDDIEQWFTEDPGPDEAPRMPEAAPPVAPAPAAPTPAAPAPAPSWPLSSSVPSQKTYQGSYGFRLGFLHSGTAKSVTCTYSPALNKMFCQLAKTCPVQLWVDSTPPPGTRVRAMAIYKQSQHMTEVVRRCPHHERCSDSDGLAPPQHLIRVEGNLRVEYLDDRNTFRHSVVVPYEPPEVGSDCTTIHYNYMCNSSCMGGMNRRPILTIITLEDSSGNLLGRNSFEVRVCACPGRDRRTEEENLRKKGEPHHELPPGSTKRALPNNTSSSPQPKKKPLDGEYFTL

SEQ ID NO: 21 - protein, 277 aa, Homo sapiens
MDDLMLSPDDIEQWFTEDPGPDEAPRMPEAAPPVAPAPAAPTPAAPAPAPSWPLSSSVPSQKTYQGSYGFRLGFLHSGTAKSVTCTYSPALNKMFCQLAKTCPVQLWVDSTPPPGTRVRAMAIYKQSQHMTEVVRRCPHHERCSDSDGLAPPQHLIRVEGNLRVEYLDDRNTFRHSVVVPYEPPEVGSDCTTIHYNYMCNSSCMGGMNRRPILTIITLEDSSGNLLGRNSFEVRVCACPGRDRRTEEENLRKKGEPHHELPPGSTKRALPNNTSSSP

SEQ ID NO: 22 - protein, 266 aa, Homo sapiens
MDDLMLSPDDIEQWFTEDPGPDEAPRMPEAAPPVAPAPAAPTPAAPAPAPSWPLSSSVPSQKTYQGSYGFRLGFLHSGTAKSVTCTYSPALNKMFCQLAKTCPVQLWVDSTPPPGTRVRAMAIYKQSQHMTEVVRRCPHHERCSDSDGLAPPQHLIRVEGNLRVEYLDDRNTFRHSVVVPYEPPEVGSDCTTIHYNYMCNSSCMGGMNRRPILTIITLEDSSGNLLGRNSFEVRVCACPGRDRRTEEENLRKKGEPHHELPPGSTK

SEQ ID NO: 23 - protein, 152 aa, Homo sapiens
MDDLMLSPDDIEQWFTEDPGPDEAPRMPEAAPPVAPAPAAPTPAAPAPAPSWPLSSSVPSQKTYQGSYGFRLGFLHSGTAKSVTCTYSPALNKMFCQLAKTCPVQLWVDSTPPPGTRVRAMAIYKQSQHMTEVVRRCPHHERCSDSDGLAPP

SEQ ID NO: 24 - protein, 106 aa, Homo sapiens
MDDLMLSPDDIEQWFTEDPGPDEAPRMPEAAPPVAPAPAAPTPAAPAPAPSWPLSSSVPSQKTYQGSYGFRLGFLHSGTAKSVTCTYSPALNKMFCQLAKTCPVQL

SEQ ID NO: 25 - protein, 209 aa, Homo sapiens
MFCQLAKTCPVQLWVDSTPPPGTRVRAMAIYKQSQHMTEVVRRCPHHERCSDSDGLAPPQHLIRVEGNLRVEYLDDRNTFRHSVVVPYEPPEVGSDCTTIHYNYMCNSSCMGGMNRRPILTIITLEDSSGNLLGRNSFEVRVCACPGRDRRTEEENLRKKGEPHHELPPGSTKRALPNNTSSSPQPKKKPLDGEYFTLQIRGRERFEMF

SEQ ID NO: 26 - protein, 198 aa, Homo sapiens
MFCQLAKTCPVQLWVDSTPPPGTRVRAMAIYKQSQHMTEVVRRCPHHERCSDSDGLAPPQHLIRVEGNLRVEYLDDRNTFRHSVVVPYEPPEVGSDCTTIHYNYMCNSSCMGGMNRRPILTIITLEDSSGNLLGRNSFEVRVCACPGRDRRTEEENLRKKGEPHHELPPGSTKRALPNNTSSSPQPKKKPLDGEYFTL

SEQ ID NO: 27 - protein, 184 aa, Homo sapiens
MFCQLAKTCPVQLWVDSTPPPGTRVRAMAIYKQSQHMTEVVRRCPHHERCSDSDGLAPPQHLIRVEGNLRVEYLDDRNTFRHSVVVPYEPPEVGSDCTTIHYNYMCNSSCMGGMNRRPILTIITLEDSSGNLLGRNSFEVRVCACPGRDRRTEEENLRKKGEPHHELPPGSTKRALPNNTSSSP

SEQ ID NO: 28 - protein, 173 aa, Homo sapiens
MFCQLAKTCPVQLWVDSTPPPGTRVRAMAIYKQSQHMTEVVRRCPHHERCSDSDGLAPPQHLIRVEGNLRVEYLDDRNTFRHSVVVPYEPPEVGSDCTTIHYNYMCNSSCMGGMNRRPILTIITLEDSSGNLLGRNSFEVRVCACPGRDRRTEEENLRKKGEPHHELPPGSTK

SEQ ID NO: 29 - protein, 59 aa, Homo sapiens
MFCQLAKTCPVQLWVDSTPPPGTRVRAMAIYKQSQHMTEVVRRCPHHERCSDSDGLAPP

SEQ ID NO: 30 - protein, 13 aa, Homo sapiens
MFCQLAKTCPVQL

SEQ ID NO: 31 - protein, 182 aa, Homo sapiens
MAIYKQSQHMTEVVRRCPHHERCSDSDGLAPPQHLIRVEGNLRVEYLDDRNTFRHSVVVPYEPPEVGSDCTTIHYNYMCNSSCMGGMNRRPILTIITLEDSSGNLLGRNSFEVRVCACPGRDRRTEEENLRKKGEPHHELPPGSTKRALPNNTSSSPQPKKKPLDGEYFTLQIRGRERFEMF

SEQ ID NO: 32 - protein, 171 aa, Homo sapiens
MAIYKQSQHMTEVVRRCPHHERCSDSDGLAPPQHLIRVEGNLRVEYLDDRNTFRHSVVVPYEPPEVGSDCTTIHYNYMCNSSCMGGMNRRPILTIITLEDSSGNLLGRNSFEVRVCACPGRDRRTEEENLRKKGEPHHELPPGSTKRALPNNTSSSPQPKKKPLDGEYFTL

SEQ ID NO: 33 - protein, 157 aa, Homo sapiens
MAIYKQSQHMTEVVRRCPHHERCSDSDGLAPPQHLIRVEGNLRVEYLDDRNTFRHSVVVPYEPPEVGSDCTTIHYNYMCNSSCMGGMNRRPILTIITLEDSSGNLLGRNSFEVRVCACPGRDRRTEEENLRKKGEPHHELPPGSTKRALPNNTSSSP

SEQ ID NO: 34 - protein, 146 aa, Homo sapiens
MAIYKQSQHMTEVVRRCPHHERCSDSDGLAPPQHLIRVEGNLRVEYLDDRNTFRHSVVVPYEPPEVGSDCTTIHYNYMCNSSCMGGMNRRPILTIITLEDSSGNLLGRNSFEVRVCACPGRDRRTEEENLRKKGEPHHELPPGSTK

SEQ ID NO: 35 - protein, 32 aa, Homo sapiens
MAIYKQSQHMTEVVRRCPHHERCSDSDGLAPP

SEQ ID NO: 36 - DNA, 1182 bp, Homo sapiens
  source 1..1182: mol_type = genomic DNA
atggaggagccgcagtcagatcctagcgtcgagccccctctgagtcaggaaacattttcagacctatggaaactacttcctgaaaacaacgttctgtcccccttgccgtcccaagcaatggatgatttgatgctgtccccggacgatattgaacaatggttcactgaagacccaggtccagatgaagctcccagaatgccagaggctgctccccccgtggcccctgcaccagcagctcctacaccggcggcccctgcaccagccccctcctggcccctgtcatcttctgtcccttcccagaaaacctaccagggcagctacggtttccgtctgggcttcttgcattctgggacagccaagtctgtgacttgcacgtactcccctgccctcaacaagatgttttgccaactggccaagacctgccctgtgcagctgtgggttgattccacacccccgcccggcacccgcgtccgcgccatggccatctacaagcagtcacagcacatgacggaggttgtgaggcgctgcccccaccatgagcgctgctcagatagcgatggtctggcccctcctcagcatcttatccgagtggaaggaaatttgcgtgtggagtatttggatgacagaaacacttttcgacatagtgtggtggtgccctatgagccgcctgaggttggctctgactgtaccaccatccactacaactacatgtgtaacagttcctgcatgggcggcatgaaccggaggcccatcctcaccatcatcacactggaagactccagtggtaatctactgggacggaacagctttgaggtgcgtgtttgtgcctgtcctgggagagaccggcgcacagaggaagagaatctccgcaagaaaggggagcctcaccacgagctgcccccagggagcactaagcgagcactgcccaacaacaccagctcctctccccagccaaagaagaaaccactggatggagaatatttcacccttcagatccgtgggcgtgagcgcttcgagatgttccgagagctgaatgaggccttggaactcaaggatgcccaggctgggaaggagccaggggggagcagggctcactccagccacctgaagtccaaaaagggtcagtctacctcccgccataaaaaactcatgttcaagacagaagggcctgactcagactga

SEQ ID NO: 37 - DNA, 1026 bp, Homo sapiens
  source 1..1026: mol_type = genomic DNA
atggaggagccgcagtcagatcctagcgtcgagccccctctgagtcaggaaacattttcagacctatggaaactacttcctgaaaacaacgttctgtcccccttgccgtcccaagcaatggatgatttgatgctgtccccggacgatattgaacaatggttcactgaagacccaggtccagatgaagctcccagaatgccagaggctgctccccccgtggcccctgcaccagcagctcctacaccggcggcccctgcaccagccccctcctggcccctgtcatcttctgtcccttcccagaaaacctaccagggcagctacggtttccgtctgggcttcttgcattctgggacagccaagtctgtgacttgcacgtactcccctgccctcaacaagatgttttgccaactggccaagacctgccctgtgcagctgtgggttgattccacacccccgcccggcacccgcgtccgcgccatggccatctacaagcagtcacagcacatgacggaggttgtgaggcgctgcccccaccatgagcgctgctcagatagcgatggtctggcccctcctcagcatcttatccgagtggaaggaaatttgcgtgtggagtatttggatgacagaaacacttttcgacatagtgtggtggtgccctatgagccgcctgaggttggctctgactgtaccaccatccactacaactacatgtgtaacagttcctgcatgggcggcatgaaccggaggcccatcctcaccatcatcacactggaagactccagtggtaatctactgggacggaacagctttgaggtgcgtgtttgtgcctgtcctgggagagaccggcgcacagaggaagagaatctccgcaagaaaggggagcctcaccacgagctgcccccagggagcactaagcgagcactgcccaacaacaccagctcctctccccagccaaagaagaaaccactggatggagaatatttcacccttcaggaccagaccagctttcaaaaagaaaattgttaa

SEQ ID NO: 38 - DNA, 1041 bp, Homo sapiens
  source 1..1041: mol_type = genomic DNA
atggaggagccgcagtcagatcctagcgtcgagccccctctgagtcaggaaacattttcagacctatggaaactacttcctgaaaacaacgttctgtcccccttgccgtcccaagcaatggatgatttgatgctgtccccggacgatattgaacaatggttcactgaagacccaggtccagatgaagctcccagaatgccagaggctgctccccccgtggcccctgcaccagcagctcctacaccggcggcccctgcaccagccccctcctggcccctgtcatcttctgtcccttcccagaaaacctaccagggcagctacggtttccgtctgggcttcttgcattctgggacagccaagtctgtgacttgcacgtactcccctgccctcaacaagatgttttgccaactggccaagacctgccctgtgcagctgtgggttgattccacacccccgcccggcacccgcgtccgcgccatggccatctacaagcagtcacagcacatgacggaggttgtgaggcgctgcccccaccatgagcgctgctcagatagcgatggtctggcccctcctcagcatcttatccgagtggaaggaaatttgcgtgtggagtatttggatgacagaaacacttttcgacatagtgtggtggtgccctatgagccgcctgaggttggctctgactgtaccaccatccactacaactacatgtgtaacagttcctgcatgggcggcatgaaccggaggcccatcctcaccatcatcacactggaagactccagtggtaatctactgggacggaacagctttgaggtgcgtgtttgtgcctgtcctgggagagaccggcgcacagaggaagagaatctccgcaagaaaggggagcctcaccacgagctgcccccagggagcactaagcgagcactgcccaacaacaccagctcctctccccagccaaagaagaaaccactggatggagaatatttcacccttcagatgctacttgacttacgatggtgttacttcctgataaactcgtcgtaa

SEQ ID NO: 39 - DNA, 1065 bp, Homo sapiens
  source 1..1065: mol_type = genomic DNA
atggatgatttgatgctgtccccggacgatattgaacaatggttcactgaagacccaggtccagatgaagctcccagaatgccagaggctgctccccccgtggcccctgcaccagcagctcctacaccggcggcccctgcaccagccccctcctggcccctgtcatcttctgtcccttcccagaaaacctaccagggcagctacggtttccgtctgggcttcttgcattctgggacagccaagtctgtgacttgcacgtactcccctgccctcaacaagatgttttgccaactggccaagacctgccctgtgcagctgtgggttgattccacacccccgcccggcacccgcgtccgcgccatggccatctacaagcagtcacagcacatgacggaggttgtgaggcgctgcccccaccatgagcgctgctcagatagcgatggtctggcccctcctcagcatcttatccgagtggaaggaaatttgcgtgtggagtatttggatgacagaaacacttttcgacatagtgtggtggtgccctatgagccgcctgaggttggctctgactgtaccaccatccactacaactacatgtgtaacagttcctgcatgggcggcatgaaccggaggcccatcctcaccatcatcacactggaagactccagtggtaatctactgggacggaacagctttgaggtgcgtgtttgtgcctgtcctgggagagaccggcgcacagaggaagagaatctccgcaagaaaggggagcctcaccacgagctgcccccagggagcactaagcgagcactgcccaacaacaccagctcctctccccagccaaagaagaaaccactggatggagaatatttcacccttcagatccgtgggcgtgagcgcttcgagatgttccgagagctgaatgaggccttggaactcaaggatgcccaggctgggaaggagccaggggggagcagggctcactccagccacctgaagtccaaaaagggtcagtctacctcccgccataaaaaactcatgttcaagacagaagggcctgactcagactga

SEQ ID NO: 40 - DNA, 909 bp, Homo sapiens
  source 1..909: mol_type = genomic DNA
atggatgatttgatgctgtccccggacgatattgaacaatggttcactgaagacccaggtccagatgaagctcccagaatgccagaggctgctccccccgtggcccctgcaccagcagctcctacaccggcggcccctgcaccagccccctcctggcccctgtcatcttctgtcccttcccagaaaacctaccagggcagctacggtttccgtctgggcttcttgcattctgggacagccaagtctgtgacttgcacgtactcccctgccctcaacaagatgttttgccaactggccaagacctgccctgtgcagctgtgggttgattccacacccccgcccggcacccgcgtccgcgccatggccatctacaagcagtcacagcacatgacggaggttgtgaggcgctgcccccaccatgagcgctgctcagatagcgatggtctggcccctcctcagcatcttatccgagtggaaggaaatttgcgtgtggagtatttggatgacagaaacacttttcgacatagtgtggtggtgccctatgagccgcctgaggttggctctgactgtaccaccatccactacaactacatgtgtaacagttcctgcatgggcggcatgaaccggaggcccatcctcaccatcatcacactggaagactccagtggtaatctactgggacggaacagctttgaggtgcgtgtttgtgcctgtcctgggagagaccggcgcacagaggaagagaatctccgcaagaaaggggagcctcaccacgagctgcccccagggagcactaagcgagcactgcccaacaacaccagctcctctccccagccaaagaagaaaccactggatggagaatatttcacccttcaggaccagaccagctttcaaaaagaaaattgttaa

SEQ ID NO: 41 - DNA, 924 bp, Homo sapiens
  source 1..924: mol_type = genomic DNA
atggatgatttgatgctgtccccggacgatattgaacaatggttcactgaagacccaggtccagatgaagctcccagaatgccagaggctgctccccccgtggcccctgcaccagcagctcctacaccggcggcccctgcaccagccccctcctggcccctgtcatcttctgtcccttcccagaaaacctaccagggcagctacggtttccgtctgggcttcttgcattctgggacagccaagtctgtgacttgcacgtactcccctgccctcaacaagatgttttgccaactggccaagacctgccctgtgcagctgtgggttgattccacacccccgcccggcacccgcgtccgcgccatggccatctacaagcagtcacagcacatgacggaggttgtgaggcgctgcccccaccatgagcgctgctcagatagcgatggtctggcccctcctcagcatcttatccgagtggaaggaaatttgcgtgtggagtatttggatgacagaaacacttttcgacatagtgtggtggtgccctatgagccgcctgaggttggctctgactgtaccaccatccactacaactacatgtgtaacagttcctgcatgggcggcatgaaccggaggcccatcctcaccatcatcacactggaagactccagtggtaatctactgggacggaacagctttgaggtgcgtgtttgtgcctgtcctgggagagaccggcgcacagaggaagagaatctccgcaagaaaggggagcctcaccacgagctgcccccagggagcactaagcgagcactgcccaacaacaccagctcctctccccagccaaagaagaaaccactggatggagaatatttcacccttcagatgctacttgacttacgatggtgttacttcctgataaactcgtcgtaa

SEQ ID NO: 42 - DNA, 786 bp, Homo sapiens
  source 1..786: mol_type = genomic DNA
atgttttgccaactggccaagacctgccctgtgcagctgtgggttgattccacacccccgcccggcacccgcgtccgcgccatggccatctacaagcagtcacagcacatgacggaggttgtgaggcgctgcccccaccatgagcgctgctcagatagcgatggtctggcccctcctcagcatcttatccgagtggaaggaaatttgcgtgtggagtatttggatgacagaaacacttttcgacatagtgtggtggtgccctatgagccgcctgaggttggctctgactgtaccaccatccactacaactacatgtgtaacagttcctgcatgggcggcatgaaccggaggcccatcctcaccatcatcacactggaagactccagtggtaatctactgggacggaacagctttgaggtgcgtgtttgtgcctgtcctgggagagaccggcgcacagaggaagagaatctccgcaagaaaggggagcctcaccacgagctgcccccagggagcactaagcgagcactgcccaacaacaccagctcctctccccagccaaagaagaaaccactggatggagaatatttcacccttcagatccgtgggcgtgagcgcttcgagatgttccgagagctgaatgaggccttggaactcaaggatgcccaggctgggaaggagccaggggggagcagggctcactccagccacctgaagtccaaaaagggtcagtctacctcccgccataaaaaactcatgttcaagacagaagggcctgactcagactga

SEQ ID NO: 43 - DNA, 630 bp, Homo sapiens
  source 1..630: mol_type = genomic DNA
atgttttgccaactggccaagacctgccctgtgcagctgtgggttgattccacacccccgcccggcacccgcgtccgcgccatggccatctacaagcagtcacagcacatgacggaggttgtgaggcgctgcccccaccatgagcgctgctcagatagcgatggtctggcccctcctcagcatcttatccgagtggaaggaaatttgcgtgtggagtatttggatgacagaaacacttttcgacatagtgtggtggtgccctatgagccgcctgaggttggctctgactgtaccaccatccactacaactacatgtgtaacagttcctgcatgggcggcatgaaccggaggcccatcctcaccatcatcacactggaagactccagtggtaatctactgggacggaacagctttgaggtgcgtgtttgtgcctgtcctgggagagaccggcgcacagaggaagagaatctccgcaagaaaggggagcctcaccacgagctgcccccagggagcactaagcgagcactgcccaacaacaccagctcctctccccagccaaagaagaaaccactggatggagaatatttcacccttcaggaccagaccagctttcaaaaagaaaattgttaa

SEQ ID NO: 44 - DNA, 645 bp, Homo sapiens
  source 1..645: mol_type = genomic DNA
atgttttgccaactggccaagacctgccctgtgcagctgtgggttgattccacacccccgcccggcacccgcgtccgcgccatggccatctacaagcagtcacagcacatgacggaggttgtgaggcgctgcccccaccatgagcgctgctcagatagcgatggtctggcccctcctcagcatcttatccgagtggaaggaaatttgcgtgtggagtatttggatgacagaaacacttttcgacatagtgtggtggtgccctatgagccgcctgaggttggctctgactgtaccaccatccactacaactacatgtgtaacagttcctgcatgggcggcatgaaccggaggcccatcctcaccatcatcacactggaagactccagtggtaatctactgggacggaacagctttgaggtgcgtgtttgtgcctgtcctgggagagaccggcgcacagaggaagagaatctccgcaagaaaggggagcctcaccacgagctgcccccagggagcactaagcgagcactgcccaacaacaccagctcctctccccagccaaagaagaaaccactggatggagaatatttcacccttcagatgctacttgacttacgatggtgttacttcctgataaactcgtcgtaa

SEQ ID NO: 45 - DNA, 705 bp, Homo sapiens
  source 1..705: mol_type = genomic DNA
atggccatctacaagcagtcacagcacatgacggaggttgtgaggcgctgcccccaccatgagcgctgctcagatagcgatggtctggcccctcctcagcatcttatccgagtggaaggaaatttgcgtgtggagtatttggatgacagaaacacttttcgacatagtgtggtggtgccctatgagccgcctgaggttggctctgactgtaccaccatccactacaactacatgtgtaacagttcctgcatgggcggcatgaaccggaggcccatcctcaccatcatcacactggaagactccagtggtaatctactgggacggaacagctttgaggtgcgtgtttgtgcctgtcctgggagagaccggcgcacagaggaagagaatctccgcaagaaaggggagcctcaccacgagctgcccccagggagcactaagcgagcactgcccaacaacaccagctcctctccccagccaaagaagaaaccactggatggagaatatttcacccttcagatccgtgggcgtgagcgcttcgagatgttccgagagctgaatgaggccttggaactcaaggatgcccaggctgggaaggagccaggggggagcagggctcactccagccacctgaagtccaaaaagggtcagtctacctcccgccataaaaaactcatgttcaagacagaagggcctgactcagactga

SEQ ID NO: 46 - DNA, 549 bp, Homo sapiens
  source 1..549: mol_type = genomic DNA
atggccatctacaagcagtcacagcacatgacggaggttgtgaggcgctgcccccaccatgagcgctgctcagatagcgatggtctggcccctcctcagcatcttatccgagtggaaggaaatttgcgtgtggagtatttggatgacagaaacacttttcgacatagtgtggtggtgccctatgagccgcctgaggttggctctgactgtaccaccatccactacaactacatgtgtaacagttcctgcatgggcggcatgaaccggaggcccatcctcaccatcatcacactggaagactccagtggtaatctactgggacggaacagctttgaggtgcgtgtttgtgcctgtcctgggagagaccggcgcacagaggaagagaatctccgcaagaaaggggagcctcaccacgagctgcccccagggagcactaagcgagcactgcccaacaacaccagctcctctccccagccaaagaagaaaccactggatggagaatatttcacccttcaggaccagaccagctttcaaaaagaaaattgttaa

SEQ ID NO: 47 - DNA, 564 bp, Homo sapiens
  source 1..564: mol_type = genomic DNA
atggccatctacaagcagtcacagcacatgacggaggttgtgaggcgctgcccccaccatgagcgctgctcagatagcgatggtctggcccctcctcagcatcttatccgagtggaaggaaatttgcgtgtggagtatttggatgacagaaacacttttcgacatagtgtggtggtgccctatgagccgcctgaggttggctctgactgtaccaccatccactacaactacatgtgtaacagttcctgcatgggcggcatgaaccggaggcccatcctcaccatcatcacactggaagactccagtggtaatctactgggacggaacagctttgaggtgcgtgtttgtgcctgtcctgggagagaccggcgcacagaggaagagaatctccgcaagaaaggggagcctcaccacgagctgcccccagggagcactaagcgagcactgcccaacaacaccagctcctctccccagccaaagaagaaaccactggatggagaatatttcacccttcagatgctacttgacttacgatggtgttacttcctgataaactcgtcgtaa

SEQ ID NO: 48 - DNA, 1026 bp, Homo sapiens
  source 1..1026: mol_type = genomic DNA
atggaggagccgcagtcagatcctagcgtcgagccccctctgagtcaggaaacattttcagacctatggaaactacttcctgaaaacaacgttctgtcccccttgccgtcccaagcaatggatgatttgatgctgtccccggacgatattgaacaatggttcactgaagacccaggtccagatgaagctcccagaatgccagaggctgctccccccgtggcccctgcaccagcagctcctacaccggcggcccctgcaccagccccctcctggcccctgtcatcttctgtcccttcccagaaaacctaccagggcagctacggtttccgtctgggcttcttgcattctgggacagccaagtctgtgacttgcacgtactcccctgccctcaacaagatgttttgccaactggccaagacctgccctgtgcagctgtgggttgattccacacccccgcccggcacccgcgtccgcgccatggccatctacaagcagtcacagcacatgacggaggttgtgaggcgctgcccccaccatgagcgctgctcagatagcgatggtctggcccctcctcagcatcttatccgagtggaaggaaatttgcgtgtggagtatttggatgacagaaacacttttcgacatagtgtggtggtgccctatgagccgcctgaggttggctctgactgtaccaccatccactacaactacatgtgtaacagttcctgcatgggcggcatgaaccggaggcccatcctcaccatcatcacactggaagactccagtggtaatctactgggacggaacagctttgaggtgcgtgtttgtgcctgtcctgggagagaccggcgcacagaggaagagaatctccgcaagaaaggggagcctcaccacgagctgcccccagggagcactaagcgagcactgcccaacaacaccagctcctctccccagccaaagaagaaaccactggatggagaatatttcacccttcagatccgtgggcgtgagcgcttcgagatgttctga

SEQ ID NO: 49 - DNA, 993 bp, Homo sapiens
  source 1..993: mol_type = genomic DNA
atggaggagccgcagtcagatcctagcgtcgagccccctctgagtcaggaaacattttcagacctatggaaactacttcctgaaaacaacgttctgtcccccttgccgtcccaagcaatggatgatttgatgctgtccccggacgatattgaacaatggttcactgaagacccaggtccagatgaagctcccagaatgccagaggctgctccccccgtggcccctgcaccagcagctcctacaccggcggcccctgcaccagccccctcctggcccctgtcatcttctgtcccttcccagaaaacctaccagggcagctacggtttccgtctgggcttcttgcattctgggacagccaagtctgtgacttgcacgtactcccctgccctcaacaagatgttttgccaactggccaagacctgccctgtgcagctgtgggttgattccacacccccgcccggcacccgcgtccgcgccatggccatctacaagcagtcacagcacatgacggaggttgtgaggcgctgcccccaccatgagcgctgctcagatagcgatggtctggcccctcctcagcatcttatccgagtggaaggaaatttgcgtgtggagtatttggatgacagaaacacttttcgacatagtgtggtggtgccctatgagccgcctgaggttggctctgactgtaccaccatccactacaactacatgtgtaacagttcctgcatgggcggcatgaaccggaggcccatcctcaccatcatcacactggaagactccagtggtaatctactgggacggaacagctttgaggtgcgtgtttgtgcctgtcctgggagagaccggcgcacagaggaagagaatctccgcaagaaaggggagcctcaccacgagctgcccccagggagcactaagcgagcactgcccaacaacaccagctcctctccccagccaaagaagaaaccactggatggagaatatttcaccctttag

SEQ ID NO: 50 - DNA, 951 bp, Homo sapiens
  source 1..951: mol_type = genomic DNA
atggaggagccgcagtcagatcctagcgtcgagccccctctgagtcaggaaacattttcagacctatggaaactacttcctgaaaacaacgttctgtcccccttgccgtcccaagcaatggatgatttgatgctgtccccggacgatattgaacaatggttcactgaagacccaggtccagatgaagctcccagaatgccagaggctgctccccccgtggcccctgcaccagcagctcctacaccggcggcccctgcaccagccccctcctggcccctgtcatcttctgtcccttcccagaaaacctaccagggcagctacggtttccgtctgggcttcttgcattctgggacagccaagtctgtgacttgcacgtactcccctgccctcaacaagatgttttgccaactggccaagacctgccctgtgcagctgtgggttgattccacacccccgcccggcacccgcgtccgcgccatggccatctacaagcagtcacagcacatgacggaggttgtgaggcgctgcccccaccatgagcgctgctcagatagcgatggtctggcccctcctcagcatcttatccgagtggaaggaaatttgcgtgtggagtatttggatgacagaaacacttttcgacatagtgtggtggtgccctatgagccgcctgaggttggctctgactgtaccaccatccactacaactacatgtgtaacagttcctgcatgggcggcatgaaccggaggcccatcctcaccatcatcacactggaagactccagtggtaatctactgggacggaacagctttgaggtgcgtgtttgtgcctgtcctgggagagaccggcgcacagaggaagagaatctccgcaagaaaggggagcctcaccacgagctgcccccagggagcactaagcgagcactgcccaacaacaccagctcctctccctag

SEQ ID NO: 51 - DNA, 918 bp, Homo sapiens
  source 1..918: mol_type = genomic DNA
atggaggagccgcagtcagatcctagcgtcgagccccctctgagtcaggaaacattttcagacctatggaaactacttcctgaaaacaacgttctgtcccccttgccgtcccaagcaatggatgatttgatgctgtccccggacgatattgaacaatggttcactgaagacccaggtccagatgaagctcccagaatgccagaggctgctccccccgtggcccctgcaccagcagctcctacaccggcggcccctgcaccagccccctcctggcccctgtcatcttctgtcccttcccagaaaacctaccagggcagctacggtttccgtctgggcttcttgcattctgggacagccaagtctgtgacttgcacgtactcccctgccctcaacaagatgttttgccaactggccaagacctgccctgtgcagctgtgggttgattccacacccccgcccggcacccgcgtccgcgccatggccatctacaagcagtcacagcacatgacggaggttgtgaggcgctgcccccaccatgagcgctgctcagatagcgatggtctggcccctcctcagcatcttatccgagtggaaggaaatttgcgtgtggagtatttggatgacagaaacacttttcgacatagtgtggtggtgccctatgagccgcctgaggttggctctgactgtaccaccatccactacaactacatgtgtaacagttcctgcatgggcggcatgaaccggaggcccatcctcaccatcatcacactggaagactccagtggtaatctactgggacggaacagctttgaggtgcgtgtttgtgcctgtcctgggagagaccggcgcacagaggaagagaatctccgcaagaaaggggagcctcaccacgagctgcccccagggagcactaagtga

SEQ ID NO: 52 - DNA, 576 bp, Homo sapiens
  source 1..576: mol_type = genomic DNA
atggaggagccgcagtcagatcctagcgtcgagccccctctgagtcaggaaacattttcagacctatggaaactacttcctgaaaacaacgttctgtcccccttgccgtcccaagcaatggatgatttgatgctgtccccggacgatattgaacaatggttcactgaagacccaggtccagatgaagctcccagaatgccagaggctgctccccccgtggcccctgcaccagcagctcctacaccggcggcccctgcaccagccccctcctggcccctgtcatcttctgtcccttcccagaaaacctaccagggcagctacggtttccgtctgggcttcttgcattctgggacagccaagtctgtgacttgcacgtactcccctgccctcaacaagatgttttgccaactggccaagacctgccctgtgcagctgtgggttgattccacacccccgcccggcacccgcgtccgcgccatggccatctacaagcagtcacagcacatgacggaggttgtgaggcgctgcccccaccatgagcgctgctcagatagcgatggtctggcccctccttag

SEQ ID NO: 53 - DNA, 438 bp, Homo sapiens
  source 1..438: mol_type = genomic DNA
atggaggagccgcagtcagatcctagcgtcgagccccctctgagtcaggaaacattttcagacctatggaaactacttcctgaaaacaacgttctgtcccccttgccgtcccaagcaatggatgatttgatgctgtccccggacgatattgaacaatggttcactgaagacccaggtccagatgaagctcccagaatgccagaggctgctccccccgtggcccctgcaccagcagctcctacaccggcggcccctgcaccagccccctcctggcccctgtcatcttctgtcccttcccagaaaacctaccagggcagctacggtttccgtctgggcttcttgcattctgggacagccaagtctgtgacttgcacgtactcccctgccctcaacaagatgttttgccaactggccaagacctgccctgtgcagctgtag

SEQ ID NO: 54 - DNA, 909 bp, Homo sapiens
  source 1..909: mol_type = genomic DNA
atggatgatttgatgctgtccccggacgatattgaacaatggttcactgaagacccaggtccagatgaagctcccagaatgccagaggctgctccccccgtggcccctgcaccagcagctcctacaccggcggcccctgcaccagccccctcctggcccctgtcatcttctgtcccttcccagaaaacctaccagggcagctacggtttccgtctgggcttcttgcattctgggacagccaagtctgtgacttgcacgtactcccctgccctcaacaagatgttttgccaactggccaagacctgccctgtgcagctgtgggttgattccacacccccgcccggcacccgcgtccgcgccatggccatctacaagcagtcacagcacatgacggaggttgtgaggcgctgcccccaccatgagcgctgctcagatagcgatggtctggcccctcctcagcatcttatccgagtggaaggaaatttgcgtgtggagtatttggatgacagaaacacttttcgacatagtgtggtggtgccctatgagccgcctgaggttggctctgactgtaccaccatccactacaactacatgtgtaacagttcctgcatgggcggcatgaaccggaggcccatcctcaccatcatcacactggaagactccagtggtaatctactgggacggaacagctttgaggtgcgtgtttgtgcctgtcctgggagagaccggcgcacagaggaagagaatctccgcaagaaaggggagcctcaccacgagctgcccccagggagcactaagcgagcactgcccaacaacaccagctcctctccccagccaaagaagaaaccactggatggagaatatttcacccttcagatccgtgggcgtgagcgcttcgagatgttctga

SEQ ID NO: 55 - DNA, 876 bp, Homo sapiens
  source 1..876: mol_type = genomic DNA
atggatgatttgatgctgtccccggacgatattgaacaatggttcactgaagacccaggtccagatgaagctcccagaatgccagaggctgctccccccgtggcccctgcaccagcagctcctacaccggcggcccctgcaccagccccctcctggcccctgtcatcttctgtcccttcccagaaaacctaccagggcagctacggtttccgtctgggcttcttgcattctgggacagccaagtctgtgacttgcacgtactcccctgccctcaacaagatgttttgccaactggccaagacctgccctgtgcagctgtgggttgattccacacccccgcccggcacccgcgtccgcgccatggccatctacaagcagtcacagcacatgacggaggttgtgaggcgctgcccccaccatgagcgctgctcagatagcgatggtctggcccctcctcagcatcttatccgagtggaaggaaatttgcgtgtggagtatttggatgacagaaacacttttcgacatagtgtggtggtgccctatgagccgcctgaggttggctctgactgtaccaccatccactacaactacatgtgtaacagttcctgcatgggcggcatgaaccggaggcccatcctcaccatcatcacactggaagactccagtggtaatctactgggacggaacagctttgaggtgcgtgtttgtgcctgtcctgggagagaccggcgcacagaggaagagaatctccgcaagaaaggggagcctcaccacgagctgcccccagggagcactaagcgagcactgcccaacaacaccagctcctctccccagccaaagaagaaaccactggatggagaatatttcaccctttag

SEQ ID NO: 56 - DNA, 834 bp, Homo sapiens
  source 1..834: mol_type = genomic DNA
atggatgatttgatgctgtccccggacgatattgaacaatggttcactgaagacccaggtccagatgaagctcccagaatgccagaggctgctccccccgtggcccctgcaccagcagctcctacaccggcggcccctgcaccagccccctcctggcccctgtcatcttctgtcccttcccagaaaacctaccagggcagctacggtttccgtctgggcttcttgcattctgggacagccaagtctgtgacttgcacgtactcccctgccctcaacaagatgttttgccaactggccaagacctgccctgtgcagctgtgggttgattccacacccccgcccggcacccgcgtccgcgccatggccatctacaagcagtcacagcacatgacggaggttgtgaggcgctgcccccaccatgagcgctgctcagatagcgatggtctggcccctcctcagcatcttatccgagtggaaggaaatttgcgtgtggagtatttggatgacagaaacacttttcgacatagtgtggtggtgccctatgagccgcctgaggttggctctgactgtaccaccatccactacaactacatgtgtaacagttcctgcatgggcggcatgaaccggaggcccatcctcaccatcatcacactggaagactccagtggtaatctactgggacggaacagctttgaggtgcgtgtttgtgcctgtcctgggagagaccggcgcacagaggaagagaatctccgcaagaaaggggagcctcaccacgagctgcccccagggagcactaagcgagcactgcccaacaacaccagctcctctccctag

SEQ ID NO: 57 - DNA, 801 bp, Homo sapiens
  source 1..801: mol_type = genomic DNA
atggatgatttgatgctgtccccggacgatattgaacaatggttcactgaagacccaggtccagatgaagctcccagaatgccagaggctgctccccccgtggcccctgcaccagcagctcctacaccggcggcccctgcaccagccccctcctggcccctgtcatcttctgtcccttcccagaaaacctaccagggcagctacggtttccgtctgggcttcttgcattctgggacagccaagtctgtgacttgcacgtactcccctgccctcaacaagatgttttgccaactggccaagacctgccctgtgcagctgtgggttgattccacacccccgcccggcacccgcgtccgcgccatggccatctacaagcagtcacagcacatgacggaggttgtgaggcgctgcccccaccatgagcgctgctcagatagcgatggtctggcccctcctcagcatcttatccgagtggaaggaaatttgcgtgtggagtatttggatgacagaaacacttttcgacatagtgtggtggtgccctatgagccgcctgaggttggctctgactgtaccaccatccactacaactacatgtgtaacagttcctgcatgggcggcatgaaccggaggcccatcctcaccatcatcacactggaagactccagtggtaatctactgggacggaacagctttgaggtgcgtgtttgtgcctgtcctgggagagaccggcgcacagaggaagagaatctccgcaagaaaggggagcctcaccacgagctgcccccagggagcactaagtga

SEQ ID NO: 58 - DNA, 459 bp, Homo sapiens
  source 1..459: mol_type = genomic DNA
atggatgatttgatgctgtccccggacgatattgaacaatggttcactgaagacccaggtccagatgaagctcccagaatgccagaggctgctccccccgtggcccctgcaccagcagctcctacaccggcggcccctgcaccagccccctcctggcccctgtcatcttctgtcccttcccagaaaacctaccagggcagctacggtttccgtctgggcttcttgcattctgggacagccaagtctgtgacttgcacgtactcccctgccctcaacaagatgttttgccaactggccaagacctgccctgtgcagctgtgggttgattccacacccccgcccggcacccgcgtccgcgccatggccatctacaagcagtcacagcacatgacggaggttgtgaggcgctgcccccaccatgagcgctgctcagatagcgatggtctggcccctccttag

SEQ ID NO: 59 - DNA, 321 bp, Homo sapiens
  source 1..321: mol_type = genomic DNA
atggatgatttgatgctgtccccggacgatattgaacaatggttcactgaagacccaggtccagatgaagctcccagaatgccagaggctgctccccccgtggcccctgcaccagcagctcctacaccggcggcccctgcaccagccccctcctggcccctgtcatcttctgtcccttcccagaaaacctaccagggcagctacggtttccgtctgggcttcttgcattctgggacagccaagtctgtgacttgcacgtactcccctgccctcaacaagatgttttgccaactggccaagacctgccctgtgcagctgtag

SEQ ID NO: 60 - DNA, 630 bp, Homo sapiens
  source 1..630: mol_type = genomic DNA
atgttttgccaactggccaagacctgccctgtgcagctgtgggttgattccacacccccgcccggcacccgcgtccgcgccatggccatctacaagcagtcacagcacatgacggaggttgtgaggcgctgcccccaccatgagcgctgctcagatagcgatggtctggcccctcctcagcatcttatccgagtggaaggaaatttgcgtgtggagtatttggatgacagaaacacttttcgacatagtgtggtggtgccctatgagccgcctgaggttggctctgactgtaccaccatccactacaactacatgtgtaacagttcctgcatgggcggcatgaaccggaggcccatcctcaccatcatcacactggaagactccagtggtaatctactgggacggaacagctttgaggtgcgtgtttgtgcctgtcctgggagagaccggcgcacagaggaagagaatctccgcaagaaaggggagcctcaccacgagctgcccccagggagcactaagcgagcactgcccaacaacaccagctcctctccccagccaaagaagaaaccactggatggagaatatttcacccttcagatccgtgggcgtgagcgcttcgagatgttctga

SEQ ID NO: 61 - DNA, 597 bp, Homo sapiens
  source 1..597: mol_type = genomic DNA
atgttttgccaactggccaagacctgccctgtgcagctgtgggttgattccacacccccgcccggcacccgcgtccgcgccatggccatctacaagcagtcacagcacatgacggaggttgtgaggcgctgcccccaccatgagcgctgctcagatagcgatggtctggcccctcctcagcatcttatccgagtggaaggaaatttgcgtgtggagtatttggatgacagaaacacttttcgacatagtgtggtggtgccctatgagccgcctgaggttggctctgactgtaccaccatccactacaactacatgtgtaacagttcctgcatgggcggcatgaaccggaggcccatcctcaccatcatcacactggaagactccagtggtaatctactgggacggaacagctttgaggtgcgtgtttgtgcctgtcctgggagagaccggcgcacagaggaagagaatctccgcaagaaaggggagcctcaccacgagctgcccccagggagcactaagcgagcactgcccaacaacaccagctcctctccccagccaaagaagaaaccactggatggagaatatttcaccctttag

SEQ ID NO: 62 - DNA, 555 bp, Homo sapiens
  source 1..555: mol_type = genomic DNA
atgttttgccaactggccaagacctgccctgtgcagctgtgggttgattccacacccccgcccggcacccgcgtccgcgccatggccatctacaagcagtcacagcacatgacggaggttgtgaggcgctgcccccaccatgagcgctgctcagatagcgatggtctggcccctcctcagcatcttatccgagtggaaggaaatttgcgtgtggagtatttggatgacagaaacacttttcgacatagtgtggtggtgccctatgagccgcctgaggttggctctgactgtaccaccatccactacaactacatgtgtaacagttcctgcatgggcggcatgaaccggaggcccatcctcaccatcatcacactggaagactccagtggtaatctactgggacggaacagctttgaggtgcgtgtttgtgcctgtcctgggagagaccggcgcacagaggaagagaatctccgcaagaaaggggagcctcaccacgagctgcccccagggagcactaagcgagcactgcccaacaacaccagctcctctccctag

SEQ ID NO: 63 - DNA, 522 bp, Homo sapiens
  source 1..522: mol_type = genomic DNA
atgttttgccaactggccaagacctgccctgtgcagctgtgggttgattccacacccccgcccggcacccgcgtccgcgccatggccatctacaagcagtcacagcacatgacggaggttgtgaggcgctgcccccaccatgagcgctgctcagatagcgatggtctggcccctcctcagcatcttatccgagtggaaggaaatttgcgtgtggagtatttggatgacagaaacacttttcgacatagtgtggtggtgccctatgagccgcctgaggttggctctgactgtaccaccatccactacaactacatgtgtaacagttcctgcatgggcggcatgaaccggaggcccatcctcaccatcatcacactggaagactccagtggtaatctactgggacggaacagctttgaggtgcgtgtttgtgcctgtcctgggagagaccggcgcacagaggaagagaatctccgcaagaaaggggagcctcaccacgagctgcccccagggagcactaagtga

SEQ ID NO: 64 - DNA, 180 bp, Homo sapiens
  source 1..180: mol_type = genomic DNA
atgttttgccaactggccaagacctgccctgtgcagctgtgggttgattccacacccccgcccggcacccgcgtccgcgccatggccatctacaagcagtcacagcacatgacggaggttgtgaggcgctgcccccaccatgagcgctgctcagatagcgatggtctggcccctccttag

SEQ ID NO: 65 - DNA, 42 bp, Homo sapiens
  source 1..42: mol_type = genomic DNA
atgttttgccaactggccaagacctgccctgtgcagctgtag

SEQ ID NO: 66 - DNA, 549 bp, Homo sapiens
  source 1..549: mol_type = genomic DNA
atggccatctacaagcagtcacagcacatgacggaggttgtgaggcgctgcccccaccatgagcgctgctcagatagcgatggtctggcccctcctcagcatcttatccgagtggaaggaaatttgcgtgtggagtatttggatgacagaaacacttttcgacatagtgtggtggtgccctatgagccgcctgaggttggctctgactgtaccaccatccactacaactacatgtgtaacagttcctgcatgggcggcatgaaccggaggcccatcctcaccatcatcacactggaagactccagtggtaatctactgggacggaacagctttgaggtgcgtgtttgtgcctgtcctgggagagaccggcgcacagaggaagagaatctccgcaagaaaggggagcctcaccacgagctgcccccagggagcactaagcgagcactgcccaacaacaccagctcctctccccagccaaagaagaaaccactggatggagaatatttcacccttcagatccgtgggcgtgagcgcttcgagatgttctga

SEQ ID NO: 67 - DNA, 516 bp, Homo sapiens
  source 1..516: mol_type = genomic DNA
atggccatctacaagcagtcacagcacatgacggaggttgtgaggcgctgcccccaccatgagcgctgctcagatagcgatggtctggcccctcctcagcatcttatccgagtggaaggaaatttgcgtgtggagtatttggatgacagaaacacttttcgacatagtgtggtggtgccctatgagccgcctgaggttggctctgactgtaccaccatccactacaactacatgtgtaacagttcctgcatgggcggcatgaaccggaggcccatcctcaccatcatcacactggaagactccagtggtaatctactgggacggaacagctttgaggtgcgtgtttgtgcctgtcctgggagagaccggcgcacagaggaagagaatctccgcaagaaaggggagcctcaccacgagctgcccccagggagcactaagcgagcactgcccaacaacaccagctcctctccccagccaaagaagaaaccactggatggagaatatttcaccctttag

SEQ ID NO: 68 - DNA, 474 bp, Homo sapiens
  source 1..474: mol_type = genomic DNA
atggccatctacaagcagtcacagcacatgacggaggttgtgaggcgctgcccccaccatgagcgctgctcagatagcgatggtctggcccctcctcagcatcttatccgagtggaaggaaatttgcgtgtggagtatttggatgacagaaacacttttcgacatagtgtggtggtgccctatgagccgcctgaggttggctctgactgtaccaccatccactacaactacatgtgtaacagttcctgcatgggcggcatgaaccggaggcccatcctcaccatcatcacactggaagactccagtggtaatctactgggacggaacagctttgaggtgcgtgtttgtgcctgtcctgggagagaccggcgcacagaggaagagaatctccgcaagaaaggggagcctcaccacgagctgcccccagggagcactaagcgagcactgcccaacaacaccagctcctctccctag

SEQ ID NO: 69 - DNA, 441 bp, Homo sapiens
  source 1..441: mol_type = genomic DNA
atggccatctacaagcagtcacagcacatgacggaggttgtgaggcgctgcccccaccatgagcgctgctcagatagcgatggtctggcccctcctcagcatcttatccgagtggaaggaaatttgcgtgtggagtatttggatgacagaaacacttttcgacatagtgtggtggtgccctatgagccgcctgaggttggctctgactgtaccaccatccactacaactacatgtgtaacagttcctgcatgggcggcatgaaccggaggcccatcctcaccatcatcacactggaagactccagtggtaatctactgggacggaacagctttgaggtgcgtgtttgtgcctgtcctgggagagaccggcgcacagaggaagagaatctccgcaagaaaggggagcctcaccacgagctgcccccagggagcactaagtga

SEQ ID NO: 70 - DNA, 99 bp, Homo sapiens
  source 1..99: mol_type = genomic DNA
atggccatctacaagcagtcacagcacatgacggaggttgtgaggcgctgcccccaccatgagcgctgctcagatagcgatggtctggcccctccttag